European Patent Specification EP 3 818 073 B1, published December 3, 2025. Title: Bakterienstamm zur Freisetzung eines rekombinanten Proteins in einem Fermentationsverfahren. Applicant: Wacker Chemie AG Koch, Dr. Johanna Brunner, Markus. The sequence listing filed with the application follows.

SEQUENCE LISTING (7 sequences)

SEQ ID NO: 1 - DNA, 816 bp, Artificial Sequence
  DNS-Fragment xI
  misc_feature (1)..(816)
caattcgcgcgcgtaacaaaagtgtctataatcacggcagaaaagtccacattgattatttgcacggcgtcacactttgctatgccatagcatttttatccataagattagcggatcctacctgacgctttttatcgcaactctctactgtttctccatacccgtttttttgggctagaaataattttgtttaagaattctaaggaggaaattatatgcaactgaacaaagtgctgaaagggctgatgattgctctgcctgttatggcaattgcggcagccagcaatgacggcagcgaaggcatgctgggtgccggcactggtatggatgcgaacggcggcaacggcaacatgtcttccgaagagcaggctcgtctgcaaatgcaacagctgcagcagaacaacatcgtttacttcgatctggacaagtacgatatccgttctgacttcgctcaaatgctggatgcacatgcaaacttcctgcgtagcaacccgtcttacaaagtcaccgtagaaggtcacgcggacgaacgtggtactccggaatacaacatctccctgggtgaacgtcgtgcgaacgccgttaagatgtacctgcagggtaaaggcgtttctgcagaccagatctccatcgtttcttacggtaaagaaaaacctgcagtactgggtcatgacgaagcggcatactccaaaaaccgtcgtgcggtactggtttactaagaattgcaagctggccgacgcgtcccacagccgccagttccgctggcggcattttaactttctttaatgaagccggaaaaatcccgcgcgcgaaggc

SEQ ID NO: 2 - DNA, 771 bp, Artificial Sequence
  DNS-Fragment xII
  misc_feature (1)..(771)
caattcgcgcgcgtaacaaaagtgtctataatcacggcagaaaagtccacattgattatttgcacggcgtcacactttgctatgccatagcatttttatccataagattagcggatcctacctgacgctttttatcgcaactctctactgtttctccatacccgtttttttgggctagaaataattttgtttaagaattctaaggaggaaattatatgaaaaagacagctatcgcgattgcagtggcactggctggtttcgctaccgtagcgcaggctgccgcagaggcagatgatattttcggtgagctaagctctggtaagaatgcaccgaaaacggggggaggggcgaaagggaacaatgcttcgcctgccgggagtggtaatactaaaaacaatggcgcatcaggggccgatatcaataactatgccgggcagattaaatctgctatcgaaagtaagttctatgacgcatcgtcctatgcaggcaaaacctgtacgctgcgcataaaactggcacccgatggtatgttactggatatcaaacctgaaggtggcgatcccgcactttgtcaggctgcgttggcagcagctaaacttgcgaagatcccgaaaccaccaagccaggcagtatatgaagtgttcaaaaacgcaccattggacttcaaaccgtaagaattgcaagctggccgacgcgtcccacagccgccagttccgctggcggcattttaactttctttaatgaagccggaaaaatcccgcgcgcgaaggc

SEQ ID NO: 3 - DNA, 1599 bp, Artificial Sequence
  DNS-Fragment xIII
  misc_feature (1)..(1599)
acagaattctaaggaggaaattatatgaaaagaaaccgtttttttaatacctcggctgctattgccatttcgattgcattacagatcttttttccgtccgcttccgctttcgctcaggttcagctggtgcagagcggtgccgaagttgttaaaccgggtgcaagcgttaaactgagctgtaaagcaagcggctatatttttaccagctattatatgtattgggtgaaacaggcaccgggtcagggtctggaatggattggtgaaattaatccgagcaatggcgataccaattttaatgaaaaatttaaaagcaaagccaccctgaccgttgataaaagcgcaagcaccgcatatatggaactgagcagcctgcgtagcgaagataccgcagtttattattgtacccgtagtgatggtcgcaatgatatggatagctggggtcagggcaccctggtcaccgttagcagcgcaagcaccaaaggtccgagcgtttttccgctggcaccgagcagcaaaagcaccagcggtggcaccgcagcactgggttgtctggttaaagattattttccggaaccggttacagttagctggaatagcggtgcactgaccagtggtgttcatacctttccggcagttctgcaaagcagcggtctgtatagcctgagcagcgttgttaccgttccgagcagtagcctgggcacccagacctatatttgtaatgttaatcataaaccgagcaacaccaaagtggataaaaaagttgaaccgaaaagctgctaataaccatggagaaaataaagtgaaacaaagcactattgcactggcactcttaccgttactcttcacccctgttaccaaagccgatattgtgctcacccagagtccggcaaccctgagcgttagtccgggtgaacgtgcaaccattagctgtcgtgcaagccagcgtgttagcagcagcacctatagctatatgcattggtatcagcagaaaccgggtcagcctccgaaactgctgattaaatatgcaagcaatctggaaagcggtgttccggcacgttttagcggtagcggtagtggcaccgattttaccctgaccattagcagcgttgaaccggaagattttgccacctattattgtcagcatagctgggaaattcctccgacctttggtggtggcaccaaactcgagattaaacgtaccgttgcagcaccgagcgtgtttatctttccgcctagtgatgaacagctgaaaagcggcaccgcaagcgttgtttgtctgctgaataacttttatccgcgtgaagcaaaagttcagtggaaagttgataatgcactgcaaagcggtaatagccaagaaagcgttaccgaacaggatagcaaagatagcacctatagcctgtcaagcaccctgaccctgagcaaagcagattatgaaaaacacaaagtgtatgcctgcgaagttacccatcagggtctgagcagtccggttacaaaaagttttaatcgtggtgaatgtagctcttctgcccatcaccaccatcaccattaataagcttctagaagcttggctgttttggcggatgagagaagattttcgac

SEQ ID NO: 4 - protein, 173 aa, Escherichia coli
  PEPTIDE (1)..(173): Wildtyp-Pal-Protein
MQLNKVLKGLMIALPVMAIAACSSNKNASNDGSEGMLGAGTGMDANGGNGNMSSEEQARLQMQQLQQNNIVYFDLDKYDIRSDFAQMLDAHANFLRSNPSYKVTVEGHADERGTPEYNISLGERRANAVKMYLQGKGVSADQISIVSYGKEKPAVLGHDEAAYSKNRRAVLVY

SEQ ID NO: 5 - protein, 167 aa, Artificial Sequence
  PalD22-27
  PEPTIDE (1)..(167)
MQLNKVLKGLMIALPVMAIAAASNDGSEGMLGAGTGMDANGGNGNMSSEEQARLQMQQLQQNNIVYFDLDKYDIRSDFAQMLDAHANFLRSNPSYKVTVEGHADERGTPEYNISLGERRANAVKMYLQGKGVSADQISIVSYGKEKPAVLGHDEAAYSKNRRAVLVY

SEQ ID NO: 6 - DNA, 834 bp, Artificial Sequence
  DNS-Fragment xIA
  misc_feature (1)..(834)
caattcgcgcgcgtaacaaaagtgtctataatcacggcagaaaagtccacattgattatttgcacggcgtcacactttgctatgccatagcatttttatccataagattagcggatcctacctgacgctttttatcgcaactctctactgtttctccatacccgtttttttgggctagaaataattttgtttaagaattctaaggaggaaattatatgcaactgaacaaagtgctgaaagggctgatgattgctctgcctgttatggcaattgcggcagcttcttccaacaagaacgccagcaatgacggcagcgaaggcatgctgggtgccggcactggtatggatgcgaacggcggcaacggcaacatgtcttccgaagagcaggctcgtctgcaaatgcaacagctgcagcagaacaacatcgtttacttcgatctggacaagtacgatatccgttctgacttcgctcaaatgctggatgcacatgcaaacttcctgcgtagcaacccgtcttacaaagtcaccgtagaaggtcacgcggacgaacgtggtactccggaatacaacatctccctgggtgaacgtcgtgcgaacgccgttaagatgtacctgcagggtaaaggcgtttctgcagaccagatctccatcgtttcttacggtaaagaaaaacctgcagtactgggtcatgacgaagcggcatactccaaaaaccgtcgtgcggtactggtttactaagaattgcaagctggccgacgcgtcccacagccgccagttccgctggcggcattttaactttctttaatgaagccggaaaaatcccgcgcgcgaaggc

SEQ ID NO: 7 - protein, 173 aa, Artificial Sequence
  Pal22A
  PEPTIDE (1)..(173)
MQLNKVLKGLMIALPVMAIAAASSNKNASNDGSEGMLGAGTGMDANGGNGNMSSEEQARLQMQQLQQNNIVYFDLDKYDIRSDFAQMLDAHANFLRSNPSYKVTVEGHADERGTPEYNISLGERRANAVKMYLQGKGVSADQISIVSYGKEKPAVLGHDEAAYSKNRRAVLVY